European Patent Application EP 4 356 757 A1, published April 24, 2024. Title: MICROBIAL METHOD FOR REPRODUCING THE HUMAN UROLITHIN METABOTYPES IN VITRO AND IN VIVO. Applicant: Consejo Superior de Investigaciones Cientificas (CSIC). Application ES. The sequence listing filed with the application follows.

SEQUENCE LISTING (9 sequences)

SEQ ID NO: 1 - DNA, 24 bp, synthetic construct
  source 1..24: mol_type = other DNA; note = Primer forward Gordonibacter; note (original language) = Cebador directo Gordonibacter; organism (original language) = construccion sintetica
ggctcgagtttggtagaggaagat

SEQ ID NO: 2 - DNA, 18 bp, synthetic construct
  source 1..18: mol_type = other DNA; note = Primer reverse Gordonibacter; note (original language) = Cebador reverso Gordonibacter; organism (original language) = construccion sintetica
ggcccagaagactgcctt

SEQ ID NO: 3 - DNA, 25 bp, synthetic construct
  source 1..25: mol_type = other DNA; note = Probe Gordonibacter; note (original language) = Sonda Gordonibacter; organism (original language) = construccion sintetica
aattcccggtgtagcggtggaatgc

SEQ ID NO: 4 - DNA, 17 bp, synthetic construct
  source 1..17: mol_type = other DNA; note = Primer forward Ellagibacter; note (original language) = Cebador directo Ellagibacter; organism (original language) = construccion sintetica
gctaggtgtggggaaac

SEQ ID NO: 5 - DNA, 17 bp, synthetic construct
  source 1..17: mol_type = other DNA; note = Primer reverse Ellagibacter; note (original language) = Cebador reverso Ellagibacter; organism (original language) = construccion sintetica
ctcaaaggaattgacgg

SEQ ID NO: 6 - DNA, 14 bp, synthetic construct
  source 1..14: mol_type = other DNA; note = Ellagibacter Probe; note (original language) = Sonda Ellagibacter; organism (original language) = construccion sintetica
tacggcggcaacgc

SEQ ID NO: 7 - DNA, 20 bp, synthetic construct
  source 1..20: mol_type = other DNA; note = Primer forward Enterocloster; note (original language) = Cebador directo Enterocloster; organism (original language) = construccion sintetica
acgtcccagttcggactgta

SEQ ID NO: 8 - DNA, 20 bp, synthetic construct
  source 1..20: mol_type = other DNA; note = Primer reverse Enterocloster; note (original language) = Cebador reverso Enterocloster; organism (original language) = construccion sintetica
gttgctgactcccatggtgt

SEQ ID NO: 9 - DNA, 24 bp, synthetic construct
  source 1..24: mol_type = other DNA; note = Probe Enterocloster; note (original language) = Sonda Enterocloster; organism (original language) = construccion sintetica
caacccgactacacgaagctggaa